European Patent Specification EP 3 659 585 B1, published June 25, 2025. Title: Composition for delivering physiologically active igredients into blood vessel. Applicant: LEMONEX INC. Application PCT/KR2018/008445. The sequence listing filed with the application follows.

SEQUENCE LISTING (10 sequences)

SEQ ID NO: 1 - RNA, 21 nt, Artificial Sequence
  GFP siRNA sense
ggcuacguccaggagcgcacc

SEQ ID NO: 2 - RNA, 21 nt, Artificial Sequence
  GFP siRNA antisense
ugcgcuccuggacguagccuu

SEQ ID NO: 3 - protein, 1386 aa, Artificial Sequence
  Cas9
MDKKYSIGLDIGTNSVGWAVITDEYKVPSKKFKVLGNTDRHSIKKNLIGALLFDSGETAEATRLKRTARRRYTRRKNRICYLQEIFSNEMAKVDDSFFHRLEESFLVEEDKKHERHPIFGNIVDEVAYHEKYPTIYHLRKKLVDSTDKADLRLIYLALAHMIKFRGHFLIEGDLNPDNSDVDKLFIQLVQTYNQLFEENPINASGVDAKAILSARLSKSRRLENLIAQLPGEKKNGLFGNLIALSLGLTPNFKSNFDLAEDAKLQLSKDTYDDDLDNLLAQIGDQYADLFLAAKNLSDAILLSDILRVNTEITKAPLSASMIKRYDEHHQDLTLLKALVRQQLPEKYKEIFFDQSKNGYAGYIDGGASQEEFYKFIKPILEKMDGTEELLVKLNREDLLRKQRTFDNGSIPHQIHLGELHAILRRQEDFYPFLKDNREKIEKILTFRIPYYVGPLARGNSRFAWMTRKSEETITPWNFEEVVDKGASAQSFIERMTNFDKNLPNEKVLPKHSLLYEYFTVYNELTKVKYVTEGMRKPAFLSGEQKKAIVDLLFKTNRKVTVKQLKEDYFKKIECFDSVEISGVEDRFNASLGTYHDLLKIIKDKDFLDNEENEDILEDIVLTLTLFEDREMIEERLKTYAHLFDDKVMKQLKRRRYTGWGRLSRKLINGIRDKQSGKTILDFLKSDGFANRNFMQLIHDDSLTFKEDIQKAQVSGQGDSLHEHIANLAGSPAIKKGILQTVKVVDELVKVMGRHKPENIVIEMARENQTTQKGQKNSRERMKRIEEGIKELGSQILKEHPVENTQLQNEKLYLYYLQNGRDMYVDQELDINRLSDYDVDHIVPQSFLKDDSIDNKVLTRSDKNRGKSDNVPSEEVVKKMKNYWRQLLNAKLITQRKFDNLTKAERGGLSELDKAGFIKRQLVETRQITKHVAQILDSRMNTKYDENDKLIREVKVITLKSKLVSDFRKDFQFYKVREINNYHHAHDAYLNAVVGTALIKKYPKLESEFVYGDYKVYDVRKMIAKSEQEIGKATAKYFFYSNIMNFFKTEITLANGEIRKRPLIETNGETGEIVWDKGRDFATVRKVLSMPQVNIVKKTEVQTGGFSKESILPKRNSDKLIARKKDWDPKKYGGFDSPTVAYSVLVVAKVEKGKSKKLKSVKELLGITIMERSSFEKNPIDFLEAKGYKEVKKDLIIKLPKYSLFELENGRKRMLASAGELQKGNELALPSKYVNFLYLASHYEKLKGSPEDNEQKQLFVEQHKHYLDEIIEQISEFSKRVILADANLDKVLSAYNKHRDKPIREQAENIIHLFTLTNLGAPAAFKYFDTTIDRKRYTSTKEVLDATLIHQSITGLYETRIDLSQLGGDGGSGPPKKKRKVHHHHHH

SEQ ID NO: 4 - RNA, 130 nt, Artificial Sequence
  Guide RNA
gaaauuaauacgacucacuauaggggcccaguggaucuaaaugagggguuuuagagcuagaaauagcaaguuaaaauaaggcuaguccguuaucaacuugaaaaaguggcaccgagucggugcuuuuuuu

SEQ ID NO: 5 - DNA, 1878 bp, Artificial Sequence
  plasmid DNA
ttcgcgatgtacgggccagatatacgcgttgacattgattattgactagttattaatagtaatcaattacggggtcattagttcatagcccatatatggagttccgcgttacataacttacggtaaatggcccgcctggctgaccgcccaacgacccccgcccattgacgtcaataatgacgtatgttcccatagtaacgccaatagggactttccattgacgtcaatgggtggagtatttacggtaaactgcccacttggcagtacatcaagtgtatcatatgccaagtacgccccctattgacgtcaatgacggtaaatggcccgcctggcattatgcccagtacatgaccttatgggactttcctacttggcagtacatctacgtattagtcatcgctattaccatggtgatgcggttttggcagtacatcaatgggcgtggatagcggtttgactcacggggatttccaagtctccaccccattgacgtcaatgggagtttgttttggcaccaaaatcaacgggactttccaaaatgtcgtaacaactccgccccattgacgcaaatgggcggtaggcgtgtacggtgggaggtctatataagcagagctcgtttagtgaaccgtcagatcgcctggagacgccatccacgctgttttgacctccatagaagacaccgggaccgatccagcctccggactctagaggatcgaacccttttggaccctcgtacagaagctaatacgactcactatagggaaataagagagaaaagaagagtaagaagaaatataagagccaccatggtgagcaagggcgaggagctgttcaccggggtggtgcccatcctggtcgagctggacggcgacgtaaacggccacaagttcagcgtgtccggcgagggcgagggcgatgccacctacggcaagctgaccctgaagttcatctgcaccaccggcaagctgcccgtgccctggcccaccctcgtgaccaccctgacctacggcgtgcagtgcttcagccgctaccccgaccacatgaagcagcacgacttcttcaagtccgccatgcccgaaggctacgtccaggagcgcaccatcttcttcaaggacgacggcaactacaagacccgcgccgaggtgaagttcgagggcgacaccctggtgaaccgcatcgagctgaagggcatcgacttcaaggaggacggcaacatcctggggcacaagctggagtacaactacaacagccacaacgtctatatcatggccgacaagcagaagaacggcatcaaggtgaacttcaagatccgccacaacatcgaggacggcagcgtgcagctcgccgaccactaccagcagaacacccccatcggcgacggccccgtgctgctgcccgacaaccactacctgagcacccagtccgccctgagcaaagaccccaacgagaagcgcgatcacatggtcctgctggagttcgtgaccgccgccgggatcactctcggcatggacgagctgtacaagtaagctgccttctgcggggcttgccttctggccatgcccttcttctctcccttgcacctgtacctcttggtctttgaataaagcctgagtaggaagtgagggtctagaactagtgtcgacgcaagggttcgatccctaccggttagtaatgagtttaaacgggggaggctaactgaaacacggaaggagacaataccggaaggaacccgcgctatgacggcaataaaaagacagaataaaacgcacgggtgttgggtcgtttgttcataaacgcggggttcggtcccagggctggcactctgtcgataccccaccgagaccccattggggccaatacgcccgcgtttcttccttt

SEQ ID NO: 6 - DNA, 1878 bp, Artificial Sequence; identical to SEQ ID NO: 5
  linear DNA

SEQ ID NO: 7 - RNA, 23 nt, Artificial Sequence
  VEGF repressing siRNA sense strand
ggaguacccugaugagaucdtdt

SEQ ID NO: 8 - RNA, 23 nt, Artificial Sequence
  VEGF repressing siRNA antisense strand
ggaguacccugaugagaucdtdt

SEQ ID NO: 9 - protein, 19 aa, Artificial Sequence
  p53 peptide
  MISC_FEATURE (1): xaa is 2-amino-5-azido-pentanoic acid
  MISC_FEATURE (4): xaa is Qln
  MISC_FEATURE (6)..(7): Xaa is Qln
  MISC_FEATURE (10): Xaa is a non-natural amino acid with introduced alkyne functional group  wherein 4-pentynoic acid is introduced on a side chain of D-Lys
  MISC_FEATURE (17): Xaa is 20amino-5-azido-pentanoic acid
  MISC_FEATURE (18): Xaa is Qln
XGGXSXXTFXNLWRLLXXN

SEQ ID NO: 10 - RNA, 191 nt, Artificial Sequence
  mRNA
  misc_feature (191): n is (Adenine) >=100
tttgttcataaacgcggggttcggtcccagggctggcactctgtcgataccccaccgagaccccattggggccaatacgcccgcgtttcttccttttccccaccccaccccccaagttcgggtgaaggcccagggctcgcagccaacgtcggggcggcaggccctgccatagcagatctgcgcagctgggn